European Patent Application EP 4 302 765 A1, published January 10, 2024. Title: Composition for preventing, alleviating, or treating Sarcopenia comprising D-ribo-2-hexulose as active ingredient. Applicant: Kyungpook National University Industry-Academic Cooperation Foundation. The sequence listing filed with the application follows.

SEQUENCE LISTING (34 sequences)

SEQ ID NO: 1 - DNA, 20 bp, Artificial Sequence
  GAPDH_F
tgcagtggcaaagtggagat

SEQ ID NO: 2 - DNA, 20 bp, Artificial Sequence
  GAPDH_R
ttgaatttgccgtgagtgga

SEQ ID NO: 3 - DNA, 24 bp, Artificial Sequence
  Atrogin-1_F
aaccgggaggccagctaaagaaca

SEQ ID NO: 4 - DNA, 23 bp, Artificial Sequence
  Atrogin-1_R
tgggcctacagaacagacagtgc

SEQ ID NO: 5 - DNA, 19 bp, Artificial Sequence
  FoxO3_F
tcgcctcctggcgggctta

SEQ ID NO: 6 - DNA, 20 bp, Artificial Sequence
  FoxO3_R
acggcggtgctagcctgaga

SEQ ID NO: 7 - DNA, 28 bp, Artificial Sequence
  Mef2_F
acacgcataatggatgagaggaaccgac

SEQ ID NO: 8 - DNA, 28 bp, Artificial Sequence
  Mef2_R
caacgatatccgagttcgtcctgctttc

SEQ ID NO: 9 - DNA, 20 bp, Artificial Sequence
  Myf5_F
aggaaaagaagccctgaagc

SEQ ID NO: 10 - DNA, 20 bp, Artificial Sequence
  Myf5_R
gcaaaaagaacaggcagagg

SEQ ID NO: 11 - DNA, 22 bp, Artificial Sequence
  Myf6_F
caagaaaatcttgagggtgcgg

SEQ ID NO: 12 - DNA, 20 bp, Artificial Sequence
  Myf6_R
ttagccgttatcacgagccc

SEQ ID NO: 13 - DNA, 20 bp, Artificial Sequence
  MyoD_F
gcttctatcgccgccactcc

SEQ ID NO: 14 - DNA, 20 bp, Artificial Sequence
  MyoD_R
cgcacatgctcatcctcacg

SEQ ID NO: 15 - DNA, 18 bp, Artificial Sequence
  Myogenin_F
ccttgctcagctccctca

SEQ ID NO: 16 - DNA, 19 bp, Artificial Sequence
  Myogenin_R
tgggagttgcattcactgg

SEQ ID NO: 17 - DNA, 20 bp, Artificial Sequence
  MuRF1_F
gagaacctggagaagcagct

SEQ ID NO: 18 - DNA, 18 bp, Artificial Sequence
  MuRF1_R
ccgcggttggtccagtag

SEQ ID NO: 19 - DNA, 17 bp, Artificial Sequence
  CerS1_F
gcagccaccacacacat

SEQ ID NO: 20 - DNA, 20 bp, Artificial Sequence
  CerS1_R
atgcctgacctccagtcata

SEQ ID NO: 21 - DNA, 20 bp, Artificial Sequence
  CIDEC_F
tccaggacatcttgaaactt

SEQ ID NO: 22 - DNA, 21 bp, Artificial Sequence
  CIDEC_R
ggcttgcaagtattcttctgt

SEQ ID NO: 23 - DNA, 22 bp, Artificial Sequence
  CISH_F
ggacatggtcctttgcgtacag

SEQ ID NO: 24 - DNA, 22 bp, Artificial Sequence
  CISH_R
ggagaacgtcttggctatgcac

SEQ ID NO: 25 - DNA, 20 bp, Artificial Sequence
  SCD1_F
tcctgctcatgtgcttcatc

SEQ ID NO: 26 - DNA, 20 bp, Artificial Sequence
  SCD1_R
ggatgttctcccgagattga

SEQ ID NO: 27 - DNA, 19 bp, Artificial Sequence
  Adipsin_F
aaccggacaacctgcaatc

SEQ ID NO: 28 - DNA, 19 bp, Artificial Sequence
  Adipsin_R
cccacgtaaccacaccttc

SEQ ID NO: 29 - DNA, 18 bp, Artificial Sequence
  Adiponectin_F
ccgttcagcattcagtgt

SEQ ID NO: 30 - DNA, 19 bp, Artificial Sequence
  Adiponectin_R
cagccttgtccttcttgta

SEQ ID NO: 31 - DNA, 21 bp, Artificial Sequence
  Haptoglobin_F
ctgtggagttgggcaatgatg

SEQ ID NO: 32 - DNA, 21 bp, Artificial Sequence
  Haptoglobin_R
aaccaagtgctccacatagcc

SEQ ID NO: 33 - DNA, 20 bp, Artificial Sequence
  Neuronatin_F
gctcatcatcggctggtaca

SEQ ID NO: 34 - DNA, 20 bp, Artificial Sequence
  Neuronatin_R
cttggcaagtgctcctctga